European Patent Specification EP 3 599 828 B1, published October 25, 2023. Title: CARBOHYDRATE PRODUCING PLANT MATERIAL. Applicant: SUN, Chuanxin. The sequence listing filed with the application follows.

SEQUENCE LISTING (119 sequences)

SEQ ID NO: 1 - DNA, 26 bp, Hordeum vulgare
aagcttgctcctgctatgagtgatct

SEQ ID NO: 2 - DNA, 28 bp, Hordeum vulgare
gtcgacttcacaattaggatgtgtgcac

SEQ ID NO: 3 - DNA, 28 bp, Hordeum vulgare
aagcttgtacacaacctttaattttctt

SEQ ID NO: 4 - DNA, 26 bp, Aequorea victoria
gtcgacatggtgagcaagggcgagga

SEQ ID NO: 5 - DNA, 28 bp, Aequorea victoria
gagctcttacttgtacagctcgtccatg

SEQ ID NO: 6 - DNA, 28 bp, Escherichia coli
aagcttaactgcatcagccgattatcat

SEQ ID NO: 7 - DNA, 26 bp, Escherichia coli
gtcgacgtggtggctagcttgtttgc

SEQ ID NO: 8 - DNA, 29 bp, Cauliflower mosaic virus
gagctccatggagtcaaagattcaaatag

SEQ ID NO: 9 - DNA, 25 bp, Cauliflower mosaic virus
gtcgacagtcccccgtgttctctcc

SEQ ID NO: 10 - DNA, 29 bp, Arabidopsis thaliana
gtcgactctcagagtttaatgaagaagcg

SEQ ID NO: 11 - DNA, 26 bp, Arabidopsis thaliana
cacgtgggcaaagacattgattattc

SEQ ID NO: 12 - DNA, 28 bp, Hordeum vulgare
gggagctctccgtagtaaaagaaacagg

SEQ ID NO: 13 - DNA, 29 bp, Hordeum vulgare
cggaattctttgtaggcgtacggtagcgg

SEQ ID NO: 14 - DNA, 28 bp, Aequorea victoria
cggaattcatggtgagcaagggcgagga

SEQ ID NO: 15 - DNA, 30 bp, Aequorea victoria
ggcacgtgttacttgtacagctcgtccatg

SEQ ID NO: 16 - DNA, 28 bp, Hordeum vulgare
gggtcgacatggttgagcctgttccagc

SEQ ID NO: 17 - DNA, 28 bp, Hordeum vulgare
aacacgtgtcatggacccatgcccaagt

SEQ ID NO: 18 - DNA, 27 bp, Hordeum vulgare
cggaattctggacccatgaccaagttc

SEQ ID NO: 19 - DNA, 28 bp, Hordeum vulgare
gggagctcgaggtaaaaccctacatcct

SEQ ID NO: 20 - DNA, 33 bp, Hordeum vulgare
ttaagctttctcatgtagtaatcatacggtggg

SEQ ID NO: 21 - DNA, 28 bp, Artificial Sequence
  Blue Fluorescent Protein (BFP)
ttaagcttatggtgagcaagggcgagga

SEQ ID NO: 22 - DNA, 31 bp, Artificial Sequence
  Blue Fluorescent Protein (BFP)
aacacgtgctatttgtacagctcgtccatgc

SEQ ID NO: 23 - DNA, 28 bp, Hordeum vulgare
gcaagctttgttgcctctcttttgtaaa

SEQ ID NO: 24 - DNA, 28 bp, Hordeum vulgare
gcaagcttggtagagtttgaaggaagta

SEQ ID NO: 25 - DNA, 28 bp, Hordeum vulgare
gcaagcttgaggtaaaaccctacatcct

SEQ ID NO: 26 - DNA, 28 bp, Hordeum vulgare
gcaagcttcccgcgacccgaggacctct

SEQ ID NO: 27 - DNA, 28 bp, Hordeum vulgare
gcaagctttggctatctctctttgttga

SEQ ID NO: 28 - DNA, 28 bp, Hordeum vulgare
aaactagttctcatgtagtaatcatacg

SEQ ID NO: 29 - DNA, 28 bp, Aequorea victoria
aaactagtatggtgagcaagggcgagga

SEQ ID NO: 30 - DNA, 28 bp, Hordeum vulgare
aactcgagatgtcccccgcgcggctgcc

SEQ ID NO: 31 - DNA, 28 bp, Hordeum vulgare
aactcgagtcatggacccatgaccaagt

SEQ ID NO: 32 - DNA, 18 bp, Hordeum vulgare
gctattcatctgctgcgg

SEQ ID NO: 33 - DNA, 18 bp, Hordeum vulgare
ccgcagcagatgaatagc

SEQ ID NO: 34 - DNA, 18 bp, Hordeum vulgare
tcctattgggctggggct

SEQ ID NO: 35 - DNA, 18 bp, Hordeum vulgare
gctcaaccataccaggcg

SEQ ID NO: 36 - DNA, 18 bp, Hordeum vulgare
gtcttccacctccagcat

SEQ ID NO: 37 - DNA, 18 bp, Hordeum vulgare
accagcagactccatttt

SEQ ID NO: 38 - DNA, 18 bp, Hordeum vulgare
cgcgggggacatggcctt

SEQ ID NO: 39 - DNA, 18 bp, Hordeum vulgare
aaggccatgacccccgcg

SEQ ID NO: 40 - DNA, 20 bp, Hordeum vulgare
tcaacctcacttacagtttg

SEQ ID NO: 41 - DNA, 20 bp, Hordeum vulgare
gtgatgctctctcaacatgc

SEQ ID NO: 42 - DNA, 21 bp, Hordeum vulgare
ttgatcttggtgttggaatca

SEQ ID NO: 43 - DNA, 20 bp, Hordeum vulgare
cccatggtttgcatttgata

SEQ ID NO: 44 - DNA, 20 bp, Hordeum vulgare
tgaatgaaaacagacctccc

SEQ ID NO: 45 - DNA, 20 bp, Hordeum vulgare
atgtaccaacttcagcaggc

SEQ ID NO: 46 - DNA, 20 bp, Hordeum vulgare
gacgaacggcacgactacta

SEQ ID NO: 47 - DNA, 20 bp, Hordeum vulgare
atagaaggaggtggacgcat

SEQ ID NO: 48 - DNA, 19 bp, Arabidopsis thaliana
cgtggtgggaagagagagc

SEQ ID NO: 49 - DNA, 24 bp, Arabidopsis thaliana
tgttgatgaagcagagtcagtaga

SEQ ID NO: 50 - DNA, 20 bp, Hordeum vulgare
agacgaggcggggtcagttg

SEQ ID NO: 51 - DNA, 19 bp, Hordeum vulgare
tccccgccgcggaaactgc

SEQ ID NO: 52 - DNA, 19 bp, Hordeum vulgare
gcggtggagagcttcggtg

SEQ ID NO: 53 - DNA, 18 bp, Hordeum vulgare
gcgctgagctgtggcacc

SEQ ID NO: 54 - DNA, 18 bp, Hordeum vulgare
tgtaccctgagcacgccg

SEQ ID NO: 55 - DNA, 18 bp, Hordeum vulgare
gccagcctccatgcttcg

SEQ ID NO: 56 - DNA, 20 bp, Hordeum vulgare
aacggacgggtcagtcatcg

SEQ ID NO: 57 - DNA, 20 bp, Hordeum vulgare
ccaccaggcccttgctcacg

SEQ ID NO: 58 - DNA, 22 bp, Hordeum vulgare
gccaagaagcgcaagaagaaga

SEQ ID NO: 59 - DNA, 21 bp, Hordeum vulgare
ggtcgaagtggttggccatga

SEQ ID NO: 60 - DNA, 20 bp, Hordeum vulgare
gcgggcgcgaggtacaaggc

SEQ ID NO: 61 - DNA, 20 bp, Hordeum vulgare
agttggtgaggagcacgggg

SEQ ID NO: 62 - DNA, 20 bp, Hordeum vulgare
ctgtactgtgtttttagcct

SEQ ID NO: 63 - DNA, 20 bp, Hordeum vulgare
gacatgacacaaaaatcgga

SEQ ID NO: 64 - DNA, 20 bp, Hordeum vulgare
cacacatggcacgccaaaac

SEQ ID NO: 65 - DNA, 20 bp, Hordeum vulgare
gtgtgtaccgtgcggttttg

SEQ ID NO: 66 - DNA, 20 bp, Hordeum vulgare
ttattttgaccatatatacg

SEQ ID NO: 67 - DNA, 20 bp, Hordeum vulgare
aataaaactggtatatatgc

SEQ ID NO: 68 - DNA, 20 bp, Artificial Sequence
  Artificial version of SP8a element in 6-SFT p
ctgtaaaaaaaatttagcct

SEQ ID NO: 69 - DNA, 20 bp, Artificial Sequence
  Artificial version of SP8a element in 6-SFT p
gacattttttttaaatcgga

SEQ ID NO: 70 - DNA, 20 bp, Artificial Sequence
  Artificial version of W-box element in 6-SFT p
ttattaaaaaaatatatacg

SEQ ID NO: 71 - DNA, 20 bp, Artificial Sequence
  Artificial version of W-box element in 6-SFT p
aataatttttttatatatgc

SEQ ID NO: 72 - DNA, 20 bp, Artificial Sequence
  Artificial version of SUREa element in 6-SFT p
caaaaatggcacgccaaaac

SEQ ID NO: 73 - DNA, 20 bp, Artificial Sequence
  Artificial version of SUREa element in 6-SFT p
gttttttccgtgcggttttg

SEQ ID NO: 74 - DNA, 20 bp, Artificial Sequence
  Artificial version of SUREa element in 6-SFT p
cacacaaaaaacgccaaaac

SEQ ID NO: 75 - DNA, 20 bp, Artificial Sequence
  Artificial version of SUREa element in 6-SFT p
gtgtgttttttgcggttttg

SEQ ID NO: 76 - DNA, 20 bp, Artificial Sequence
  Artificial version of SUREa element in 6-SFT p
cacacatggcaaaaaaaaac

SEQ ID NO: 77 - DNA, 20 bp, Artificial Sequence
  Artificial version of SUREa element in 6-SFT p
gtgtgtaccgtttttttttg

SEQ ID NO: 78 - DNA, 20 bp, Artificial Sequence
  Artificial version of SUREa element in 6-SFT p
caaaaaaaaaaaaaaaaaac

SEQ ID NO: 79 - DNA, 20 bp, Artificial Sequence
  Artificial version of SUREa element in 6-SFT p
gttttttttttttttttttg

SEQ ID NO: 80 - DNA, 27 bp, Hordeum vulgare
gtacacaacctttaattttcttttctg

SEQ ID NO: 81 - DNA, 27 bp, Hordeum vulgare
catgtgttggaaattaaaagaaaagac

SEQ ID NO: 82 - DNA, 30 bp, Hordeum vulgare
tgtcctatagagattaatgcactttatctt

SEQ ID NO: 83 - DNA, 30 bp, Hordeum vulgare
acaggatatctctaattacgtgaaatagaa

SEQ ID NO: 84 - DNA, 30 bp, Hordeum vulgare
gcagaacattaagatgaaatttaagcattt

SEQ ID NO: 85 - DNA, 30 bp, Hordeum vulgare
cgtcttgtaattctactttaaattcgtaaa

SEQ ID NO: 86 - DNA, 30 bp, Hordeum vulgare
tgtttctagatgaccctgcaactttttttg

SEQ ID NO: 87 - DNA, 30 bp, Hordeum vulgare
acaaagatctactgggacgttgaaaaaaac

SEQ ID NO: 88 - DNA, 30 bp, Hordeum vulgare
gcctttattgtgcatattatataatttggc

SEQ ID NO: 89 - DNA, 30 bp, Hordeum vulgare
cggaaataacacgtataatatattaaaccg

SEQ ID NO: 90 - DNA, 30 bp, Hordeum vulgare
caggttcttgaattgttgcataattcataa

SEQ ID NO: 91 - DNA, 30 bp, Hordeum vulgare
gtccaagaacttaacaacgtattaagtatt

SEQ ID NO: 92 - DNA, 355 bp, Hordeum vulgare
gttgcctctcttttgtaaatgtatctatgagttacatattttattctgatattttttggatgataggaaggtaacgctattccagatgcatggcaaatctcaatataaaactcattaactcaatattcatgtgcagcattacttctttcacatgttgtggagaagtttctttataaatggtagagtttgaaggaagtattttgaatggcagtttggggaaaacctatggtacatatgtagttagatctatctgtgcttgctatattagtcacatcctttcttaattcgttgacttgtttttacatatttagttttgcattgtgtaacatttgtgatgtcatattttgtactgcag

SEQ ID NO: 93 - DNA, 398 bp, Oryza sativa
atttccttgctaggtgagacttgagtggtgctagtctggctgcaaatttatagaagtatgtgaaaatttgaggtcagaatacaagtaattgaatggaccaatctaatgagttctgtagctttagaataattaatgttaacataaaaatatgttcatgaaatcaggtccttctgcattttgttgttaaccgaattccacattcttctttagttctcacaagtacagacaagtatcttgtaatggtggattcttttttggaaaacaaacttcattacatattttgtgtgatccatctatgccttgtgcccttgttacctttttttccctacaccttgttttctcttgtacttagttttgcattgtataaccttttgctgtactcgtgtcttgtactgtag

SEQ ID NO: 94 - DNA, 178 bp, Hordeum vulgare
gtacacaacctttaattttcttttctgtgtcctatagagattaatgcactttatcttgcagaacattaagatgaaatttaagcattttgtttctagatgaccctgcaactttttttggcctttattgtgcatattatataatttggccaggttcttgaattgttgcataattcataat

SEQ ID NO: 95 - DNA, 605 bp, Oryza sativa
gtatggatcctttctttgagtgattacctggtatcgtgtaattcttcatttgtgtatactgtatttgagagtttgaaaaaatttccatagaaaataataacatttgttgtttacaaatggtcccgccaaaacagtggaatttatattggggatgtacataaaaggagtgtaaagttctaatgtgcttatgctaacttcctttccatgatctaaagttgttaccttacggtatgctatttattggatctatattgcattttacttggtaaatctatctgaggttccagcttttgatatttaagttttcctatgtttaattcaaaatattctcacgtgaatcgcaaacctcaccaggagtacaataaattcgttttattattattgtaggctgtgttatttctagtccatggttcggtgtcttgaaatttcagtgccaaaattgggatggatctggttacatcttcaagtctaataaatgatcacaccgactttattgtgtgatttgattatagcagggtcttgcaacataaatacaagctattaattgtgaaaggagaaatgagatctttggtgagatcatgagaatagggtataacagacacaat

SEQ ID NO: 96 - DNA, 911 bp, Hordeum vulgare
gtacacaacctttaattttcttttctgtgtcctatagagattaatgcactttatcttgcagaacattaagatgaaatttaagcattttgtttctagatgaccctgcaactttttttggcctttattgtgcatattatataatttggccaggttcttgaattgttgcataattcataatgttgcctctcttttgtaaatgtatctatgagttacatattttattctgatattttttggatgataggaaggtaacgctattccagatgcatggcaaatctcaatataaaactcattaactcaatattcatgtgcagcattacttctttcacatgttgtggagaagtttctttataaatggtagagtttgaaggaagtattttgaatggcagtttggggaaaacctatggtacatatgtagttagatctatctgtgcttgctatattagtcacatcctttcttaattcgttgacttgtttttacatatttagttttgcattgtgtaacatttgtgatgtcatattttgtactgcaggctcctgctatgagtgatctaaaaaaacatgagcattctatgcaaaatcagagtatgaatcccagctcatcatctagcaatatggtgaatgaaaacagacctccctgttcacgtgagtcgagtcttacagtgaatgtaagtgctcagaaccaacctgttggaatggttggtttgactgacagcatgcctgctgaagttggtacatctgagccgcagcagatgaatagctctgacaatgccatgcaagagccgcagtctgaaaatgttgctgacaagtcggcagatgatggctacaactggcggaaatacgggcagaagcatgtcaagggaagtgaaaaccctagaagttactacaagtgcacacatcctaattgtgaa

SEQ ID NO: 97 - DNA, 1384 bp, Oryza sativa
gtatggatcctttctttgagtgattacctggtatcgtgtaattcttcatttgtgtatactgtatttgagagtttgaaaaaatttccatagaaaataataacatttgttgtttacaaatggtcccgccaaaacagtggaatttatattggggatgtacataaaaggagtgtaaagttctaatgtgcttatgctaacttcctttccatgatctaaagttgttaccttacggtatgctatttattggatctatattgcattttacttggtaaatctatctgaggttccagcttttgatatttaagttttcctatgtttaattcaaaatattctcacgtgaatcgcaaacctcaccaggagtacaataaattcgttttattattattgtaggctgtgttatttctagtccatggttcggtgtcttgaaatttcagtgccaaaattgggatggatctggttacatcttcaagtctaataaatgatcacaccgactttattgtgtgatttgattatagcagggtcttgcaacataaatacaagctattaattgtgaaaggagaaatgagatctttggtgagatcatgagaatagggtataacagacacaatatttccttgctaggtgagacttgagtggtgctagtctggctgcaaatttatagaagtatgtgaaaatttgaggtcagaatacaagtaattgaatggaccaatctaatgagttctgtagctttagaataattaatgttaacataaaaatatgttcatgaaatcaggtccttctgcattttgttgttaaccgaattccacattcttctttagttctcacaagtacagacaagtatcttgtaatggtggattcttttttggaaaacaaacttcattacatattttgtgtgatccatctatgccttgtgcccttgttacctttttttccctacaccttgttttctcttgtacttagttttgcattgtataaccttttgctgtactcgtgtcttgtactgtaggcttctgctatcaatgatcccaaaaagcatgaaacttctatgaaaaatgaaagcctgaatactgccctgtcatctgacgatatgatgatcgacaatatacctctatgttctcgtgagtcaactctcgcagtcaatatttcaagtgccccgagccaactggttggaatggttggtttaactgacagctcacctgctgaagttggtacatctgagttgcatcagatgaatagctctggaaatgctatgcaggagtcacagcctgaaagtgtggctgaaaagtctgcagaggatggttataactggcgcaaatatgggcaaaagcatgttaagggaagtgagaacccgagaagctattacaagtgcacacatcctaactgtgat

SEQ ID NO: 98 - DNA, 181 bp, Hordeum vulgare
cttccaggttgaaccttcaccaacaactggtagtctgggcatggctgcgattctgcacaagagcgctcatccagacatgctgccttcgccacgggataaatctgttcgtaatgcccatgaagataggggttctagggattttgaattcaagcctcatctgaattcgtcttctcaatcactg

SEQ ID NO: 99 - DNA, 541 bp, Hordeum vulgare
gctcctgctatgagtgatctaaaaaaacatgagcattctatgcaaaatcagagtatgaatcccagctcatcatctagcaatatggtgaatgaaaacagacctccctgttcacgtgagtcgagtcttacagtgaatgtaagtgctcagaaccaacctgttggaatggttggtttgactgacagcatgcctgctgaagttggtacatctgagccgcagcagatgaatagctctgacaatgccatgcaagagccgcagtctgaaaatgttgctgacaagtcggcagatgatggctacaactggcggaaatacgggcagaagcatgtcaagggaagtgaaaaccctagaagttactacaagtgcacacatcctaattgtgaagtaaaaaagctattggagcgtgcagttgatggtctgatcacggaagttgtctataagggacgccacaatcatcctaagccccagcccaataggaggttagctggtggtgcagttccttcaaaccagggtgaagaacgatatgacggcgcttcagctgctgatg

SEQ ID NO: 100 - DNA, 533 bp, Hordeum vulgare
gtacacaacctttaattttcttttctgtgtcctatagagattaatgcactttatcttgcagaacattaagatgaaatttaagcattttgtttctagatgaccctgcaactttttttggcctttattgtgcatattatataatttggccaggttcttgaattgttgcataattcataatgttgcctctcttttgtaaatgtatctatgagttacatattttattctgatattttttggatgataggaaggtaacgctattccagatgcatggcaaatctcaatataaaactcattaactcaatattcatgtgcagcattacttctttcacatgttgtggagaagtttctttataaatggtagagtttgaaggaagtattttgaatggcagtttggggaaaacctatggtacatatgtagttagatctatctgtgcttgctatattagtcacatcctttcttaattcgttgacttgtttttacatatttagttttgcattgtgtaacatttgtgatgtcatattttgtactgcag

SEQ ID NO: 101 - DNA, 181 bp, Oryza sativa
tgtttaggttgaaccctctccgacaactggtactctgagcatggctgcaattatgaacaagagtgcaaatccagacatacttccttcgcctagggataaaacatctggtagcacccatgaagatggtggctctcgagattttgaattcaagcctcatctgaattcatcctctcaatcgacg

SEQ ID NO: 102 - DNA, 544 bp, Oryza sativa
gcttctgctatcaatgatcccaaaaagcatgaaacttctatgaaaaatgaaagcctgaatactgccctgtcatctgacgatatgatgatcgacaatatacctctatgttctcgtgagtcaactctcgcagtcaatatttcaagtgccccgagccaactggttggaatggttggtttaactgacagctcacctgctgaagttggtacatctgagttgcatcagatgaatagctctggaaatgctatgcaggagtcacagcctgaaagtgtggctgaaaagtctgcagaggatggttataactggcgcaaatatgggcaaaagcatgttaagggaagtgagaacccgagaagctattacaagtgcacacatcctaactgtgatgtaaaaaagctattggagcgttcgcttgatggtcagattactgaagtggtttataaagggcgtcacaatcaccctaagccccaacccaataggaggctgtctgccggtgcagttcctccaatccagggtgaagaaagatatgatggtgtggcaactactgatg

SEQ ID NO: 103 - DNA, 1003 bp, Oryza sativa
gtatggatcctttctttgagtgattacctggtatcgtgtaattcttcatttgtgtatactgtatttgagagtttgaaaaaatttccatagaaaataataacatttgttgtttacaaatggtcccgccaaaacagtggaatttatattggggatgtacataaaaggagtgtaaagttctaatgtgcttatgctaacttcctttccatgatctaaagttgttaccttacggtatgctatttattggatctatattgcattttacttggtaaatctatctgaggttccagcttttgatatttaagttttcctatgtttaattcaaaatattctcacgtgaatcgcaaacctcaccaggagtacaataaattcgttttattattattgtaggctgtgttatttctagtccatggttcggtgtcttgaaatttcagtgccaaaattgggatggatctggttacatcttcaagtctaataaatgatcacaccgactttattgtgtgatttgattatagcagggtcttgcaacataaatacaagctattaattgtgaaaggagaaatgagatctttggtgagatcatgagaatagggtataacagacacaatatttccttgctaggtgagacttgagtggtgctagtctggctgcaaatttatagaagtatgtgaaaatttgaggtcagaatacaagtaattgaatggaccaatctaatgagttctgtagctttagaataattaatgttaacataaaaatatgttcatgaaatcaggtccttctgcattttgttgttaaccgaattccacattcttctttagttctcacaagtacagacaagtatcttgtaatggtggattcttttttggaaaacaaacttcattacatattttgtgtgatccatctatgccttgtgcccttgttacctttttttccctacaccttgttttctcttgtacttagttttgcattgtataaccttttgctgtactcgtgtcttgtactgtag

SEQ ID NO: 104 - protein, 573 aa, Hordeum vulgare
MSPARLPISRESCLTIPAGFSPSALLDSPVLLTNFKVEPSPTTGSLGMAAILHKSAHPDMLPSPRDKSVRNAHEDRGSRDFEFKPHLNSSSQSLAPAMSDLKKHEHSMQNQSMNPSSSSSNMVNENRPPCSRESSLTVNVSAQNQPVGMVGLTDSMPAEVGTSEPQQMNSSDNAMQEPQSENVADKSADDGYNWRKYGQKHVKGSENPRSYYKCTHPNCEVKKLLERAVDGLITEVVYKGRHNHPKPQPNRRLAGGAVPSNQGEERYDGASAADDKSSNALSNLANPVHSPGMVEPVPASVSDDDIDAGGGRPYPGDDATEEEDLESKRRKMESAGIDAALMGKPNREPRVVVQTVSEVDILDDGYRWRKYGQKVVKGNPNPRSYYKCTSTGCPVRKHVERASHDPKSVITTYEGKHNHEVPAARNATHEMSAPPMKNVVHQINSNMPSSIGGMMRACEARNYTNQYSQAAETDTVSLDLGVGISPNHSDATNQMQSSGPDQMQYQMQTMGSMYGNMRHPSSMAAPAVQGNSAARMYGSREEKGNEGFTFRATPMDHSANLCYSSAGNLVMGP

SEQ ID NO: 105 - protein, 618 aa, Oryza sativa
MADSPNPSSGDHPAGVGGSPEKQPPVDRRVAALAAGAAGAGARYKAMSPARLPISREPCLTIPAGFSPSALLESPVLLTNFKVEPSPTTGTLSMAAIMNKSANPDILPSPRDKTSGSTHEDGGSRDFEFKPHLNSSSQSTASAINDPKKHETSMKNESLNTALSSDDMMIDNIPLCSRESTLAVNISSAPSQLVGMVGLTDSSPAEVGTSELHQMNSSGNAMQESQPESVAEKSAEDGYNWRKYGQKHVKGSENPRSYYKCTHPNCDVKKLLERSLDGQITEVVYKGRHNHPKPQPNRRLSAGAVPPIQGEERYDGVATTDDKSSNVLSILGNAVHTAGMIEPVPGSASDDDNDAGGGRPYPGDDAVEDDDLESKRRKMESAAIDAALMGKPNREPRVVVQTVSEVDILDDGYRWRKYGQKVVKGNPNPRSYYKCTNTGCPVRKHVERASHDPKSVITTYEGKHNHEVPASRNASHEMSTPPMKPVVHPINSNMQGLGGMMRACEPRTFPNQYSQAAESDTISLDLGVGISPNHSDATNQLQSSVSDQMQYQMQPMGSVYSNMGLPAMAMPTMAGNAASNIYGSREEKPSEGFTFKATPMDHSANLCYSTAGNLVMGP

SEQ ID NO: 106 - protein, 281 aa, Hordeum vulgare
MVEPVPASVSDDDIDAGGGRPYPGDDATEEEDLESKRRKMESAGIDAALMGKPNREPRVVVQTVSEVDILDDGYRWRKYGQKVVKGNPNPRSYYKCTSTGCPVRKHVERASHDPKSVITTYEGKHNHEVPAARNATHEMSAPPMKNVVHQINSNMPSSIGGMMRACEARNYTNQYSQAAETDTVSLDLGVGISPNHSDATNQMQSSGPDQMQYQMQTMGSMYGNMRHPSSMAAPAVQGNSAARMYGSREEKGNEGFTFRATPMDHSANLCYSSAGNLVMGP

SEQ ID NO: 107 - protein, 279 aa, Oryza sativa
MIEPVPGSASDDDNDAGGGRPYPGDDAVEDDDLESKRRKMESAAIDAALMGKPNREPRVVVQTVSEVDILDDGYRWRKYGQKVVKGNPNPRSYYKCTNTGCPVRKHVERASHDPKSVITTYEGKHNHEVPASRNASHEMSTPPMKPVVHPINSNMQGLGGMMRACEPRTFPNQYSQAAESDTISLDLGVGISPNHSDATNQLQSSVSDQMQYQMQPMGSVYSNMGLPAMAMPTMAGNAASNIYGSREEKPSEGFTFKATPMDHSANLCYSTAGNLVMGP

SEQ ID NO: 108 - DNA, 30 bp, Hordeum vulgare
taggtcgtcaatttgacttatataaaatat

SEQ ID NO: 109 - DNA, 30 bp, Hordeum vulgare
atattttatataagtcaaattgacgaccta

SEQ ID NO: 110 - DNA, 30 bp, Hordeum vulgare
gcttcatcaacgtatccgcacgttacacgg

SEQ ID NO: 111 - DNA, 30 bp, Hordeum vulgare
ccgtgtaacgtgcggatacgttgatgaagc

SEQ ID NO: 112 - DNA, 359 bp, Triticum aestivum
cttgcctatcatttgtaaatgcatgtacgaacttacctattttattctgatcttctttggagggtaggaaggtaacactatcccagatgcatggcaaatctcagtatagaactcattaactcaatatccatatgtaacattacttctttcacatgtagcggagaagtttctttataaatagtagagtttgaaaaaagcactttgaatgacagtttggggaaaaactatggtacatatgtagttagatctatctgtgcttgctatgttagtcacattctttcttaattcctgttgacttgtttttgcatattttgttttgcatcgtgtaacatttgtaatgctcatattttgtactgcag

SEQ ID NO: 113 - DNA, 184 bp, Triticum aestivum
gtacacaacctttaattttcttttctctgtgtcccatagagattaatgtactttatcttgcagaacatcaaaagaaaatttaagcattttgtttctatacgaccccacaaatatatctggcctttattgtgcatattataaccataattcggctaggttcttgaattgttgcataattcataat

SEQ ID NO: 114 - DNA, 2354 bp, Hordeum vulgare
agatcatgcatcgttgagccgcttggtgggcgagacggctcgatgggctccccgagcgggcacgcgggctcgatgaagtactccccgtgcttcacttctgcgccacggtgatctccttgggtcgggtccaagccgaaacctagctccggggacctcccctcgcccgccgggagctcgcccgagaagccctaccccgcggatcgacgcgtcgcggcgctcgccggcgcgggcgcgaggtacaaggccatgtcccccgcgcggctgccgatctcgcgcgagtcctgcctcaccatccccgccggcttcagcccctcagcgctcctcgactcccccgtgctcctcaccaacttcaaggttgaaccttcaccaacaactggtagtctgggcatggctgcgattctgcacaagagcgctcatccagacatgctgccttcgccacgggataaatctgttcgtaatgcccatgaagataggggttctagggattttgaattcaagcctcatctgaattcgtcttctcaatcactggctcctgctatgagtgatctaaaaaaacatgagcattctatgcaaaatcagagtatgaatcccagctcatcatctagcaatatggtgaatgaaaacagacctccctgttcacgtgagtcgagtcttacagtgaatgtaagtgctcagaaccaacctgttggaatggttggtttgactgacagcatgcctgctgaagttggtacatctgagccgcagcagatgaatagctctgacaatgccatgcaagagccgcagtctgaaaatgttgctgacaagtcggcagatgatggctacaactggcggaaatacgggcagaagcatgtcaagggaagtgaaaaccctagaagttactacaagtgcacacatcctaattgtgaagtaaaaaagctattggagcgtgcagttgatggtctgatcacggaagttgtctataagggacgccacaatcatcctaagccccagcccaataggaggttagctggtggtgcagttccttcaaaccagggtgaagaacgatatgacggcgcttcagctgctgatgataaatcttccaatgctcttagcaaccttgctaatccggtacattcgcctggtatggttgagcctgttccagcttcagttagtgatgatgacatcgatgctggaggtggaagaccctaccctggggatgatgctactgaggaggaggatttagagtcgaaacgcaggaaaatggagtctgctggtattgatgctgctctgatgggtaaacctaaccgtgagccccgtgtcgtcgttcaaactgtaagtgaggttgacatcttggatgatggctatcgttggcggaaatatggacagaaagttgtcaaaggaaaccccaatccacggagttactacaaatgcacaagcacaggatgccctgtgaggaagcatgttgagagagcatcacacgatcctaaatcagtgataacaacgtatgaaggaaaacataaccatgaagtccctgctgcgaggaatgcaacccatgagatgtccgcgcctcccatgaagaacgtcgtgcatcagattaacagcaatatgcccagcagcattggtggcatgatgagggcatgtgaagccaggaactacaccaaccaatattctcaggcggctgaaaccgacactgtcagtcttgatcttggtgttggaatcagcccaaaccacagcgacgcgacaaaccaaatgcagtcttcaggtcctgaccagatgcagtatcaaatgcaaaccatgggttcgatgtacggcaacatgagacatccatcatcaatggcagcgccagcggtacaaggaaactctgctgcccgcatgtatggttcgagagaagagaaaggtaacgaagggtttactttcagagccacaccgatggaccattcagctaacctatgctatagcagtgctgggaacttggtcatgggtccatgagagggaatgagagtgtctgcaaatgctcatagctccatgaatcatatattaccaacaatgctttgtaatgacaatctcttcagcaagattctcaattgtctcaattgtgtatcggttacaagtcagttcagccggaggcaagtatgctagtataagctatacgtgggggcactgcagcaaatacgcatgtgtctttttaagtgcggaaaaggcccttgctgtatgtagcatcgcagccctacattcgttgtacagcgaacctaatatgattaattaattagattatgagaatttggtttcgtgaactgtctaatcttctgtactggaatattgatagaaatatagattatggtaattttctttaaaaaaaaaaaaaaaaaaaaaaa

SEQ ID NO: 115 - DNA, 1074 bp, Hordeum vulgare
gtacacaacctttaattttcttttctgtgtcctatagagattaatgcactttatcttgcagaacattaagatgaaatttaagcattttgtttctagatgaccctgcaactttttttggcctttattgtgcatattatataatttggccaggttcttgaattgttgcataattcataatgttgcctctcttttgtaaatgtatctatgagttacatattttattctgatattttttggatgataggaaggtaacgctattccagatgcatggcaaatctcaatataaaactcattaactcaatattcatgtgcagcattacttctttcacatgttgtggagaagtttctttataaatggtagagtttgaaggaagtattttgaatggcagtttggggaaaacctatggtacatatgtagttagatctatctgtgcttgctatattagtcacatcctttcttaattcgttgacttgtttttacatatttagttttgcattgtgtaacatttgtgatgtcatattttgtactgcaggctcctgctatgagtgatctaaaaaaacatgagcattctatgcaaaatcagagtatgaatcccagctcatcatctagcaatatggtgaatgaaaacagacctccctgttcacgtgagtcgagtcttacagtgaatgtaagtgctcagaaccaacctgttggaatggttggtttgactgacagcatgcctgctgaagttggtacatctgagccgcagcagatgaatagctctgacaatgccatgcaagagccgcagtctgaaaatgttgctgacaagtcggcagatgatggctacaactggcggaaatacgggcagaagcatgtcaagggaagtgaaaaccctagaagttactacaagtgcacacatcctaattgtgaagtaaaaaagctattggagcgtgcagttgatggtctgatcacggaagttgtctataagggacgccacaatcatcctaagccccagcccaataggaggttagctggtggtgcagttccttcaaaccagggtgaagaacgatatgacggcgcttcagctgctgatg

SEQ ID NO: 116 - DNA, 18 bp, Hordeum vulgare
agccccagcccaatagga

SEQ ID NO: 117 - DNA, 18 bp, Hordeum vulgare
cgcctggtatggttgagc

SEQ ID NO: 118 - DNA, 18 bp, Hordeum vulgare
atgctggaggtggaagac

SEQ ID NO: 119 - DNA, 18 bp, Hordeum vulgare
aaaatggagtctgctggt